European Patent Application EP 4 748 938 A1, published May 27, 2026. Title: 一种创制广谱抗病转基因玉米的方法. Applicant: 安徽荃银高科种业股份有限公司. The sequence listing filed with the application follows.

SEQUENCE LISTING (2 sequences)

SEQ ID NO: 1 - DNA, 513 bp, synthetic construct
  source 1..513: mol_type = other DNA
atggcttcccctgcttcctctgcggttatcttcttcttcgccgtggctgctctgatgtccctgctggctatgcctgccctcgctgccagccagctcaacgctggccaaaccctcggcaccggccaatccctcgctcaaggccccaaccagttcatcatccagaacgactgcaacctcgtcctgtacgctagcaacaaggccgtctgggctacgggcaccaacggcaaggctagcggctgcgtcctcaggatgcagcgcgacggcaacctcgtcatctacagcggctccaaggtcatctgggctagcaacaccaacaggcgcgacgacaactactacctcctgctccaaagggaccgcaacgtcgtgatctacgactccagcaacaacgctatctggtccaccggcaccaacctcggcaacgcggctgttaccgtcatcccccacagcaacggcacggcggcggcttcgggcgctgctcagaacaaggtgaacgagtacctcaggccatgatga

SEQ ID NO: 2 - DNA, 12907 bp, synthetic construct
  source 1..12907: mol_type = other DNA
ccagccagccaacagctccccgaccggcagctcggcacaaaatcaccactcgatacaggcagcccatcagtccgggacggcgtcagcgggagagccgttgtaaggcggcagactttgctcatgttaccgatgctattcggaagaacggcaactaagctgccgggtttgaaacacggatgatctcgcggagggtagcatgttgattgtaacgatgacagagcgttgctgcctgtgatcaccgcggtttcaaaatcggctccgtcgatactatgttatacgccaactttgaaaacaactttgaaaaagctgttttctggtatttaaggttttagaatgcaaggaacagtgaattggagttcgtcttgttataattagcttcttggggtatctttaaatactgtagaaaagaggaaggaaataataaatggctaaaatgagaatatcaccggaattgaaaaaactgatcgaaaaataccgctgcgtaaaagatacggaaggaatgtctcctgctaaggtatataagctggtgggagaaaatgaaaacctatatttaaaaatgacggacagccggtataaagggaccacctatgatgtggaacgggaaaaggacatgatgctatggctggaaggaaagctgcctgttccaaaggtcctgcactttgaacggcatgatggctggagcaatctgctcatgagtgaggccgatggcgtcctttgctcggaagagtatgaagatgaacaaagccctgaaaagattatcgagctgtatgcggagtgcatcaggctctttcactccatcgacatatcggattgtccctatacgaatagcttagacagccgcttagccgaattggattacttactgaataacgatctggccgatgtggattgcgaaaactgggaagaagacactccatttaaagatccgcgcgagctgtatgattttttaaagacggaaaagcccgaagaggaacttgtcttttcccacggcgacctgggagacagcaacatctttgtgaaagatggcaaagtaagtggctttattgatcttgggagaagcggcagggcggacaagtggtatgacattgccttctgcgtccggtcgatcagggaggatatcggggaagaacagtatgtcgagctattttttgacttactggggatcaagcctgattgggagaaaataaaatattatattttactggatgaattgttttagtacctagaatgcatgaccaaaatcccttaacgtgagttttcgttccactgagcgtcagaccccgtagaaaagatcaaaggatcttcttgagatcctttttttctgcgcgtaatctgctgcttgcaaacaaaaaaaccaccgctaccagcggtggtttgtttgccggatcaagagctaccaactctttttccgaaggtaactggcttcagcagagcgcagataccaaatactgtccttctagtgtagccgtagttaggccaccacttcaagaactctgtagcaccgcctacatacctcgctctgctaatcctgttaccagtggctgctgccagtggcgataagtcgtgtcttaccgggttggactcaagacgatagttaccggataaggcgcagcggtcgggctgaacggggggttcgtgcacacagcccagcttggagcgaacgacctacaccgaactgagatacctacagcgtgagctatgagaaagcgccacgcttcccgaagggagaaaggcggacaggtatccggtaagcggcagggtcggaacaggagagcgcacgagggagcttccagggggaaacgcctggtatctttatagtcctgtcgggtttcgccacctctgacttgagcgtcgatttttgtgatgctcgtcaggggggcggagcctatggaaaaacgccagcaacgcggcctttttacggttcctggccttttgctggccttttgctcacatgttctttcctgcgttatcccctgattctgtggataaccgtattaccgcctttgagtgagctgataccgctcgccgcagccgaacgaccgagcgcagcgagtcagtgagcgaggaagcggaagagcgcctgatgcggtattttctccttacgcatctgtgcggtatttcacaccgcatatggtgcactctcagtacaatctgctctgatgccgcatagttaagccagtatacactccgctatcgctacgtgactgggtcatggctgcgccccgacacccgccaacacccgctgacgcgccctgacgggcttgtctgctcccggcatccgcttacagacaagctgtgaccgtctccgggagctgcatgtgtcagaggttttcaccgtcatcaccgaaacgcgcgaggcagggtgccttgatgtgggcgccggcggtcgagtggcgacggcgcggcttgtccgcgccctggtagattgcctggccgtaggccagccatttttgagcggccagcggccgcgatcctacaaggtagaatccgcctgagtcgcaagggtgacttcgcctatattggacgacggcgcgcagagggcgacctctttttgggttacgattgtaggattatcactaaaacaatacatgaacatattcaaatggcaatctctctaaggcattggaaataaatacaaataacagttgggtggagtttttcgacctgagggcgttaaccttctgttaacctaaaagctcttgcccaaacagcagaatcggcgctaattgccagcggcggaacttttccagtttcgcgaaaaatatcgccactggcaaggaatgggtttgagatggcgaagtctgtcctaaaagcagcgcctgtagttgtagggttgacggccttgatggagcgtcatgccgatgccctctcgagccaacttcaagcacatcatcttaaggttttcccgccgcattccgagaagggcattcgaacattcgggccatcggaggcgtccaagctgctcggcgttggcgagtcatatttacggcagaccgcgtctgagatgccagagttgaatgttagcatgagcccgggtggcaggcgaatgttctcaattgaagatatccatgtgattcggaagtatatggatcaggtcggccgcgggaaccggcgctacctgccacatcgtcgaggcggcgagcagcttcaggttatctctgtgatgaatttcaaaggtgggtcgggtaagaccaccaccgccgcgcatctggcgcagtacctcgctatgcgcggatatcgagtcttggccattgatctcgatcctcaagcgagcctttctgcactctttgggagccaaccggagacggacgttggcccgaacgaaacgctctacggcgctataaggtatgatgatgagcaggtggcaatcgaacgagtcgtccgagggacttacattcccgacctccacctgattcctggtaaccttgagctgatggagtttgaacacgatacgccacgcgcgctgatgaaccgcaaagagggcgacacgctcttttatggtcgcatcagccaagtaattgaagatatcgcggataactatgacgtcgtggtcatcgactgccctccccagcttgggtatctcacgctatccgcattgactgcggcgacgtccattcttgtcacggtccatccgcagatgctggatgtgatgtcgatgaaccagtttctggcaatgacatcgaaccttttgcgtgaaatcgagaatgctggcgccaagttcaagtttaattggatgcgctatctgataacccgtttcgaaccgagcgacggaccacagaaccaaatggtaggttatctgcggtcgatttttggcgaaaatgtcctcaattttccgatgcttaaaaccaccgcggtttcggacgctggcctgacaaaccagactctattcgaagtggagcgtggcctgttcacgcgctcgacctatgatcgagccttggaggcgatgaacgccgtcaacgacgagatcgaaacactgatcaaaaaagcatggggtaggcccacatgagccggaagcacatccttggcgtctcaactgacgcccctgagacgtcgcccgccgacaataggacggcaaagaaccgctccatgccgctcctcggcgtaacaaggaaggagcgcgatccggcaacgaagctcacagcgaacattggtaacgcactgcgagagcaaaacgatcgtcttagccgtgccgaagagatcgagcggcgtctcgctgaaggtcaggcagtgatagagttggatgcctcgtcaatagaaccgtctttcgtgcaggatcgtatgcgaggggacattgacgggctccttacttcgatccgggaacaaggacagcaagtcccaatccttgtgcgaccgcatccgagccagccgggccgatatcaggttgccttcggccaccgccggctacgcgccgtttcagaactcggacttccggtcagagcggtcgttcgcgaactgacggacgagcaagtggtcgtagcacagggtcaggaaaacaatgagcgcgaagatcttaccttcatcgaaaaggcgcgcttcgcacatcgcctgaacaggcagttttctcgagagattgtcatcgccgcgatgtcgatcgacaagagcaatttgtccaagatgcttctgctcgtcgacgccctcccctctgaactgaccgatgctattggtgccgctcctggtgttggacggccgagttggcaacaacttgccgagctgattgagaaagtttcttcaccggccgacgtggctaaatatgctatgtcggaggaagttcaagcgctgccatcggcagaacgattcaaggcggtgatcgctagtctgaagcccagtcgggttgcgcgtggacttcccgaggtcatggccaccccagacggcaccagaattgcacaggtgacgcagagcaaggccaaactggaaatcacgattgacaggaaggcgacgcccgattttgcgaccttcgtgctcgatcatgtgccagcgctgtatcaagcgtaccacgctgagaaccaacggaaacggggagagtaaaccgcaaaagaaaagagccccctcaacgtcgccgtcgcggaagcccttctgtctctctagcgcgaacagaatcgcatttcctcgaatcctcgtcaagagtttttagcgccgttttggtgagctgatttcctttgcctgctgaaaggtgaaagatgatgcagacaggaagtgtaacgacgccattcgggcggcggccaatgacgcttgcgcttgtgcggcgccagacggcgctggccgatatcaaacaaggcaagacagcggacaagtggaaggtctttagagacgcgtccgcggccatggaactacttggaatccagtccaacagtcttgccgtccttgatgcgctattgagctttcacccggaaacggagttgcgtcaggaggcacagctgatcgtcttcccgtcgaatgctcagcttgcccttcgggcgcatgggatggctggcgcgactttgcgtaggcacatcgccatgctcgtggagtcaggcttgatcgtccggaaggatagcgccaacggaaagcgttacgctcgtaaggatggcgctggtcagatcgagcgcgcgtttggcttcgatttgtctccgcttctcgcgcggtccgaagagctagcgatgatggcacagcaggtgatggccgatcgagcagcattcaggatggccaaagaaagtctgacgatttgccgacgggacgttcggaagctaattacggcagctatggaagagggagcggagggcgactggcaagctgtcgaggaagtctatgtggaacttgtgggtagaattccacgcgccccgacgcttgctgatgtagagtcaattctcgaagagatgtggatgctccaggaagagataatcaaccggttggaaattagagacaattcagaaaataatagcaccaatgctgcccagagcgagcagcacatacagaattcaaaacccgaatccgttaatgaacttgaacctcgctctgaaaaggagcagggcgctaagccgagtgaaatagaccgggcaaggagcgagccgataaaagcgttccccctcgggatgatcctgaaagcatgcccgaccattggcaattatgggccgagcggtgcggttgctagctggcgtgacctcatgtcggctgcggtggtggttcggtctatgctgggggtcagcccgtcggcttaccaagacgcgtgtgaggcaatgggaccggagaatgcggcagcagcgatggcgtgcattttggagcgagcgaacttcatcaattcgcccgggggctatctccgagatctgacacggcggagcgagctcgggaagttttcacttggcccgatgataatggcgctcttgaaggctagcgggcaggggacgttgcggtttggctagaattagcgagtatggagcaggatggtctgtggtcagctgaccacagacctaataggttgaaaacatgagcgttttttggatgatcgacagaccatccgattcccggagtaccaagcgtgctctgatgggagcgataacattactcaacaagcacgaaggccccatgccgatcgttgatcgtgaaggagagcctgctctacatgcggcggtattttgccggccgaggcatgtagtcgcggagcactgcctatttactgccctaggcacaaacgttgactcttggatcgagctggcagacaaagcaataacccacacagaggacgattaatggctgacgaagagatccagaatccgccggacggtactgctgctgccgaagttgagccggctgctcctagaggtagaagagcaaagaaagcaccagccgaaacagcccgcacgggatcgttcaaatccgtgaagccgaaaacccgcggcctcagcaaccgagaaaaactggagaagatcggtcaaatcgaagctcaggtcgctggcggcgcaaccttgaaggacgccgttaagatcgtgggtatttccgttcagacctattatcaatggaagagagctgcggttcaacctgtctcacagaatccggccgtgtctgtttcagttgacgatgaactcggcgagttcatccaactcgaggaggaaaatcggcggctcagaaagctggccagggcgtcggcctcggtcaatgcgtcctcacggaaggcaccgcgccgcctggcctcggtgggcgtcacttcctcgctgcgctcaagtgcgcggtacagggtcgagcgatgcacgccaagcagtgcagccgcctctttcacggtgcggccttcctggtcgatcagctcgcgggcgtgcgcgatctgtgccggggtgagggtagggcgggggccaaacttcacgcctcgggccttggcggcctcgcgcccgctccgggtgcggtcgatgattagggaacgctcgaactcggcaatgccggcgaacacggtcaacaccatgcggccggccggcgtggtggtgtcggcccacggctctgccaggctacgcaggcccgcgccggcctcctggatgcgctcggcaatgtccagtaggtcgcgggtgctgcgggccaggcggtctagcctggtcactgtcacaacgtcgccagggcgtaggtggtcaagcatcctggccagctccgggcggtcgcgcctggtgccggtgatcttctcggaaaacagcttggtgcagccggccgcgtgcagttcggcccgttggttggtcaagtcctggtcgtcggtgctgacgcgggcatagcccagcaggccagcggcggcgctcttgttcatggcgtaatgtctccggttctagtcgcaagtattctactttatgcgactaaaacacgcgacaagaaaacgccaggaaaagggcagggcggcagcctgtcgcgtaacttaggacttgtgcgacatgtcgttttcagaagacggctgcactgaacgtcagaagccgactgcactatagcagcggaggggttggatcaaagtactttgatcccgaggggaaccctgtggttggcatgcacatacaaatggacgaacggataaaccttttcacgcccttttaaatatccgattattctaataaacgctcttttctcttaggtttacccgccaatatatcctgtcaaacactgatagtttaaactgaaggcgggaaacgacaatctgatcatgagcggagaattaagggagtcacgttatgacccccgccgatgacgcgggacaagccgttttacgtttggaactgacagaaccgcaacgttgaaggagccactcagcaagctggtacgattgtaatacgactcactatagggcgaattgagcgctgtttaaacgctcttcaactggaagagcggttacgctgtttaaacgctcttcaactggaagagcggttactaccggttcactagctagctgctaatcgagctagttaccctatgaggtgacatgaagcgctcacggttactatgacggttagcttcacgactgttggtggcagtagcgtacgacttagctatagttccggacttacccttaagcgatttaaatcctgaggatatcgctatcaactttgtatagaaaagttgggccgaggtcgtgcccctctctagagataatgagcattgcatgtctaagttataaaaaattaccacatattttttttgtcacacttgtttgaagtgcagtttatctatctttatacatatatttaaactttactctacgaataatataatctatagtactacaataatatcagtgttttagagaatcatataaatgaacagttagacatggtctaaaggacaattgagtattttgacaacaggactctacagttttatctttttagtgtgcatgtgttctcctttttttttgcaaatagcttcacctatataatacttcatccattttattagtacatccatttagggtttagggttaatggtttttatagactaatttttttagtacatctattttattctattttagcctctaaattaagaaaactaaaactctattttagtttttttatttaataatttagatataaaatagaataaaataaagtgactaaaaattaaacaaataccctttaagaaattaaaaaaactaaggaaacatttttcttgtttcgagtagataatgccagcctgttaaacgccgtcgacgagtctaacggacaccaaccagcgaaccagcagcgtcgcgtcgggccaagcgaagcagacggcacggcatctctgtcgctgcctctggacccctctcgagagttccgctccaccgttggacttgctccgctgtcggcatccagaaattgcgtggcggagcggcagacgtgagccggcacggcaggcggcctcctcctcctctcacggcaccggcagctacgggggattcctttcccaccgctccttcgctttcccttcctcgcccgccgtaataaatagacaccccctccacaccctctttccccaacctcgtgttgttcggagcgcacacacacacaaccagatctcccccaaatccacccgtcggcacctccgcttcaaggtacgccgctcgtcctcccccccccccctctctaccttctctagatcggcgttccggtccatggttagggcccggtagttctacttctgttcatgtttgtgttagatccgtgtttgtgttagatccgtgctgctagcgttcgtacacggatgcgacctgtacgtcagacacgttctgattgctaacttgccagtgtttctctttggggaatcctgggatggctctagccgttccgcagacgggatcgatttcatgattttttttgtttcgttgcatagggtttggtttgcccttttcctttatttcaatatatgccgtgcacttgtttgtcgggtcatcttttcatgcttttttttgtcttggttgtgatgatgtggtctggttgggcggtcgttctagatcggagtagaattctgtttcaaactacctggtggatttattaattttggatctgtatgtgtgtgccatacatattcatagttacgaattgaagatgatggatggaaatatcgatctaggataggtatacatgttgatgcgggttttactgatgcatatacagagatgctttttgttcgcttggttgtgatgatgtggtgtggttgggcggtcgttcattcgttctagatcggagtagaatactgtttcaaactacctggtgtatttattaattttggaactgtatgtgtgtgtcatacatcttcatagttacgagtttaagatggatggaaatatcgatctaggataggtatacatgttgatgtgggttttactgatgcatatacatgatggcatatgcagcatctattcatatgctctaaccttgagtacctatctattataataaacaagtatgttttataattattttgatcttgatatacttggatgatggcatatgcagcagctatatgtggatttttttagccctgccttcatacgctatttatttgcttggtactgtttcttttgtcgatgctcaccctgttgtttggtgttacttctgcagatggcttcccctgcttcctctgcggttatcttcttcttcgccgtggctgctctgatgtccctgctggctatgcctgccctcgctgccagccagctcaacgctggccaaaccctcggcaccggccaatccctcgctcaaggccccaaccagttcatcatccagaacgactgcaacctcgtcctgtacgctagcaacaaggccgtctgggctacgggcaccaacggcaaggctagcggctgcgtcctcaggatgcagcgcgacggcaacctcgtcatctacagcggctccaaggtcatctgggctagcaacaccaacaggcgcgacgacaactactacctcctgctccaaagggaccgcaacgtcgtgatctacgactccagcaacaacgctatctggtccaccggcaccaacctcggcaacgcggctgttaccgtcatcccccacagcaacggcacggcggcggcttcgggcgctgctcagaacaaggtgaacgagtacctcaggccatgatgaagacttgtccatcttctggattggccaacttaattaatgtatgaaataaaaggatgcacacatagtgacatgctaatcactataatgtgggcatcaaagttgtgtgttatgtgtaattactagttatctgaataaaagagaaagagatcatccatatttcttatcctaaatgaatgtcacgtgtctttataattctttgatgaaccagatgcatttcattaaccaaatccatatacatataaatattaatcatatataattaatatcaattgggttagcaaaacaaatctagtctaggtgtgttttgcgaatgcggccggtccgatgtgagacttttcaacaaagggtaatatccggaaacctcctcggattccattgcccagctatctgtcactttattgtgaagatagtggaaaaggaaggtggctcctacaaatgccatcattgcgataaaggaaaggccatcgttgaagatgcctctgccgacagtggtcccaaagatggacccccacccacgaggagcatcgtggaaaaagaagacgttccaaccacgtcttcaaagcaagtggattgatgtgatatctccactgacgtaagggatgacgcacaatcccactatccttcgcaagacccttcctctatataaggaagttcatttcatttggagaggacactctagacagaaaaatttgctacattgtttcacaaacttcaaatattattcatttatttgtcagctttcaaactctttgtttcttgtttgttgattctcgagatgagcccagaacgacgcccggccgacatccgccgtgccaccgaggcggacatgccggcggtctgcaccatcgtcaaccactacatcgagacaagcacggtcaacttccgtaccgagccgcaggaaccgcaggagtggacggacgacctcgtccgtctgcgggagcgctatccctggctcgtcgccgaggtggacggcgaggtcgccggcatcgcctacgcgggcccctggaaggcacgcaacgcctacgactggacggccgagtcgaccgtgtacgtctccccccgccaccagcggacgggactgggctccacgctctacacccacctgctgaagtccctggaggcacagggcttcaagagcgtggtcgctgtcatcgggctgcccaacgacccgagcgtgcgcatgcacgaggcgctcggatatgccccccgcggcatgctgcgggcggccggcttcaagcacgggaactggcatgacgtgggtttctggcagctggacttcagcctgccggtaccgccccgtccggtcctgcccgtcaccgagatttgactcgaggatcgttcaaacatttggcaataaagtttcttaagattgaatcctgttgccggtcttgcgatgattatcatataatttctgttgaattacgttaagcatgtaataattaacatgtaatgcatgacgttatttatgagatgggtttttatgattagagtcccgcaattatacatttaatacgcgatagaaaacaaaatatagcgcgcaaactaggataaattatcgcgcgcggtgtcatctatgttactagatcgccaccgcggtggagctcgaattccggtccgaagcttaagccatggcccgggaatcttagcggccgcctgcagagttaacggcgcgccgactagctagctaaggtaccgagctcgaattcattccgattaatcgtggcctcttgctcttcaggatgaagagctatgtttaaacgtgcaagcgctactagacaattcagtacattaaaaacgtccgcaatgtgttattaagttgtctaagcgtcaatttgtttacaccacaatatatcctgcca